European Patent Application EP 4 445 723 A1, published October 16, 2024. Title: METHODS AND COMPOSITIONS FOR PERONOSPORA RESISTANCE IN SPINACH. Applicant: Seminis Vegetable Seeds, Inc. The sequence listing filed with the application follows.

SEQUENCE LISTING (9 sequences)

SEQ ID NO: 1 - DNA, 301 bp, Spinacia tetrandra
  source 1..301: mol_type = genomic DNA
attatctaaatctgccnctnttttgttngtttttggtcttgatatctatggnttggtatnggcgtatagnctagtggatagtanttgatttgcctgcatgtgggnaanntcaggtttgtttagtcaatacttatccttgaagcntnnatgrtctgcaaaaacttggtcaacttggcaagggtttgcttatgntaaagttgtatttcttaacatgncatgctaagtgttctgcactncgaagtactgtatttaggaagaaantggtgctnnaaaatgttgggnnttagaggtattgggtttg

SEQ ID NO: 2 - DNA, 301 bp, Spinacia tetrandra
  source 1..301: mol_type = genomic DNA
taaattaacaattcactggaatttgtgtattcaatgatgtaaattaaannnnttnctgctaagtttangaaataaccttgtaaaattcgtcagcttctgctgtaggcaccatgtgtatcggcaaggcctttggnccatagaaggtcaaccktgtaaaagggagaacctnaaatattaagancnagaagcnnntnngtcatgcaagatnnnncatnacagtttcattcacaannnnaanaannnnnntatgaatcataaacctttaaaatatcaactctgacaagaccaccccagaaaatng

SEQ ID NO: 3 - DNA, 301 bp, Spinacia tetrandra
  source 1..301: mol_type = genomic DNA
catcaacttcctgaatctgcaanggagctccacanccataacaacaatcaactgaactcaatgtcttaatngacccagntagcttctctttcttcttcctcttcttcttattngctgcaataaccatntttgaagcctcnttagcttgatrgtgctccangaanatctnccnccgggtcggagcagctgcnccagcgccntcatcttcagaacccgaaccnggaatatgggtcggagcgttttgggnatttncatggatttgtgggtctgaatttggtgctgctgctgctctgcatttgat

SEQ ID NO: 4 - DNA, 301 bp, Spinacia tetrandra
  source 1..301: mol_type = genomic DNA
ttcatgcccacgacatcgtgctctgccgggccacactttttcacgcccgtgacgggccatgttttttttgtatcgagcccatagacattcagacggactacctgaaatcatcngttngaacttcaaagaaagagtccgngtnaaaggatcktttctcctattaaaacgcaatccattggccgtnaaatcctcattccaccaaactgannnnnnntattttcccaaattaccctttntctctctatctctttctctcncctcttcaaacgctatacatttccctttcaatcatccatcatca

SEQ ID NO: 5 - DNA, 301 bp, Spinacia tetrandra
  source 1..301: mol_type = genomic DNA
gnncgtgttcaggtctaantttttgantcagntatttnacataaaaatttatgattttgacnnaaaatgaagtgtcgtacctacgtacaangttaaggatgnganncgtgtatntnaggtagaatgaaangtacaagtaattagaagaatkaccatactgantcannacatatntcaggttagccaanntaactatncaggtcaatatttaagccattctaaaacgtggcnnttcttatcgttgcattctttagttctactataagtatgggcagactaacaatatctgcaagttggtttt

SEQ ID NO: 6 - DNA, 301 bp, Spinacia tetrandra
  source 1..301: mol_type = genomic DNA
actgtattatcaattcaacttctgatnnnnnnnnnnnnnnnnttattaagntctgtctcccaaatctgaactcgcctgtatgtaaggcagcaggcaagcacagaatnnttgtnaccttagacttaaagatggcngtgtgcctaaacgggcyggacncatgccaagcccaatnngcatngtgcngggncgggccaaatagttcaaaacngggctcatgcacacgggttgtcaggtcgggctgctgtgtctaagcttaatttaactaaatttagtgtgttttgtcgtgtcgtgtcgggtagag

SEQ ID NO: 7 - DNA, 301 bp, Spinacia tetrandra
  source 1..301: mol_type = genomic DNA
nnatgaactcntttactttgatgattcaatggtggcttcttcnttagaagcctttgaagatgggccccttaanggtttctccgtcgaccggttngtncccggncagcagctnaaggtgtttggnnggaggaaacaacnncnntcgccgccrccttccacctcctccnccggtaataattaanctcaacactttacttttagtccaatgttgttgcataatgcatatatatgatcatatgttaatttnnnnnnnnnntttttttncccctagattttaatgagagaatcccctttgcaattg

SEQ ID NO: 8 - DNA, 301 bp, Spinacia tetrandra
  source 1..301: mol_type = genomic DNA
ggcttctcncttccggtgaattccttgagcttcgatacagataatgcgagatctgaannnnnnaanattttaggnaaataaataagatttcgaaacacacgaagtcgtataagattcagcattagaatgaaggagaaataacaaacctatyaatggttttaatgcttcttgngcatcgagatcgtgtttagaagcatcaggctcntattgctcaatgtatactctnactgttgcacctgcagaaccagtaccctgcaaaacaagagacggtattcatttcgggccgtccaaacagtggcag

SEQ ID NO: 9 - DNA, 301 bp, Spinacia tetrandra
  source 1..301: mol_type = genomic DNA
gcccctaanaaaacaattacgaaactgtatcgtttngngtttgtgattcaaatatatcttatcagttngtcaggttgttttcttnattttgtacttcatgcaatttggttcgnnnattattagcagggtgatttaagcgtntttcagacakctaagcttanaaaannnaaaangacgatattntctccaagcggtcctaaaaagaatnnnaataaatgatgtcatgatggcccctaataaaaactgnatcgtttcgcgnttgtnattcaaatatatcttatcaatttgacatgttgntttc